European Patent Specification EP 3 445 847 B1, published June 5, 2024. Title: IMMUNOMODULATORY IL2R FUSION PROTIENS AND USES THEROF. Applicant: Fred Hutchinson Cancer Research Center Schmitt, Thomas M. Greenberg, Philip D. Stromnes, Ingunn M. Cheng, Laurence. Application PCT. The sequence listing filed with the application follows.

SEQUENCE LISTING (23 sequences)

SEQ ID NO: 1 - protein, 435 aa, Artificial Sequence
  Fusion protein
MLLLVTSLLLCELPHPAFLLIPEKSDLRTVAPASSLNVRFDSRTMNLSWDCQENTTFSKCFLTDKKNRVVEPRLSNNECSCTFREICLHEGVTFEVHVNTSQRGFQQKLLYPNSGREGTAAQNFSCFIYNADLMNCTWARGPTAPRDVQYFLYIRNSKRRREIRCPYYIQDSGTHVGCHLDNLSGLTSRNYFLVNGTSREIGIQFFDSLLDTKKIERFNPPSNVTVRCNTTHCLVRWKQPRTYQKLSYLDFQYQLDVHRKNTQPGTENLLINVSGDLENRYNFPSSEPRAKHSVKIRAADVRILNWSSWSEAIEFGSDDGPFLFALEAVVISVGSMGLIISLLCVYFWLERTMPRIPTLKNLEDLVTEYHGNFSAWSGVSKGLAESLQPDYSERLCLVSEIPPKGGALGEGPGASPCNQHSPYWAPPCYTLKPET

SEQ ID NO: 2 - protein, 749 aa, Artificial Sequence
  Fusion protein
MVLAQGLLSMALLALCWERSLAGAEETIPLQTLRCYNDYTSHITCRWADTQDAQRLVNVTLIRRVNEDLLEPVSCDLSDDMPWSACPHPRCVPRRCVIPCQSFVVTDVDYFSFQPDRPLGTRLTVTLTQHVQPPEPRDLQISTDQDHFLLTWSVALGSPQSHWLSPGDLEFEVVYKRLQDSWEDAAILLSNTSQATLGPEHLMPSSTYVARVRTRLAPGSRLSGRPSKWSPEVCWDSQPGDEAQPQNLECFFDGAAVLSCSWEVRKEVASSVSFGLFYKPSPDAGEEECSPVLREGLGSLHTRHHCQIPVPDPATHGQYIVSVQPRRAEKHIKSSVNIQMAPPSLNVTKDGDSYSLRWETMKMRYEHIDHTFEIQYRKDTATWKDSKTETLQNAHSMALPALEPSTRYWARVRVRTSRTGYNGIWSEWSEARSWDTESIPWLGHLLVGLSGAFGFIILVYLLINCRNTGPWLKKVLKCNTPDPSKFFSQLSSEHGGDVQKWLSSPFPSSSFSPGGLAPEISPLEVLERDKVTQLLLQQDKVPEPASLSSNHSLTSCFTNQGYFFFHLPDALEIEACQVYFTYDPYSEEDPDEGVAGAPTGSSPQPLQPLSGEDDAYCTFPSRDDLLLFSPSLLGGPSPPSTAPGGSGAGEERMPPSLQERVPRDWDPQPLGPPTPGVPDLVDFQPPPELVLREAGEEVPDAGPREGVSFPWSRPPGQGEFRALNARLPLNTDAYLSLQELQGQDPTHLV

SEQ ID NO: 3 - protein, 441 aa, Artificial Sequence
  Fusion protein
MTSSHAMNITPLAQLALLFSTLLLPGTQALLAPTTPDAGSALNLTFDPWTRTLTWACDTAAGNVTVTSCTVTSREAGIHRRVSPFGCRCWFRRMMALHHGVTLDVNGTVGGAAAHWRLSFVNEGAAGSGAENLTCEIRAARFLSCAWREGPAAPADVRYSLRVLNSTGHDVARCMADPGDDVITQCIANDLSLLGSEAYLVVTGRSGAGPVRFLDDVVATKALERLGPPRDVTASCNSSHCTVSWAPPSTWASLTARDFQFEVQWQSAEPGSTPRKVLVVEETRLAFPSPAPHGGHKVKVRAGDTRMKHWGEWSPAHPLEAEDTRVPPSLFALEAVLIPVGTMGLIITLIFVYCWLERMPPIPPIKNLEDLVTEYQGNFSAWSGVSKGLTESLQPDYSERFCHVSEIPPKGGALGEGPGGSPCSLHSPYWPPPCYSLKPEA

SEQ ID NO: 4 - protein, 740 aa, Artificial Sequence
  Fusion protein
MDQQMALTWGLCYMALVALCWGHGVTEAEETVPLKTLQCYNDYTNHIICSWADTEDAQGLINMTLYHQLEKKQPVSCELSEELMWSECPSSHRCVPRRCVIPYTRFSITNEDYYSFRPDSDLGIQLMVPLAQNVQPPLPKNVSISSSEDRFLLEWSVSLGDAQVSWLSSKDIEFEVAYKRLQDSWEDAYSLHTSKFQVNFEPKLFLPNSIYAARVRTRLSPGSSLSGRPSRWSPEVHWDSQPGDKAQPQNLQCFFDGIQSLHCSWEVWTQTTGSVSFGLFYRPSPVAPEEKCSPVVKEPPGASVYTRYHCSLPVPEPSAHSQYTVSVKHLEQGKFIMSYNHIQMEPPTLNLTKNRDSYSLHWETQKMAYSFIEHTFQVQYKKKSDSWEDSKTENLDRAHSMDLSQLEPDTSYCARVRVKPISNYDGIWSKWSEEYTWKTDWILPMSWLRYLLLVLGCFSGFFSCVYILVKCRYLGPWLKTVLKCHIPDPSEFFSQLSSQHGGDLQKWLSSPVPLSFFSPSGPAPEISPLEVLDGDSKAVQLLLLQKDSAPLPSPSGHSQASCFTNQGYFFFHLPNALEIESCQVYFTYDPCVEEEVEEDGSRLPEGSPHPPLLPLAGEQDDYCAFPPRDDLLLFSPSLSTPNTAYGGSRAPEERSPLSLHEGLPSLASRDLMGLQRPLERMPEGDGEGLSANSSGEQASVPEGNLHGQDQDRGQGPILTLNTDAYLSLQELQAQDSVHLI

SEQ ID NO: 5 - protein, 1203 aa, Artificial Sequence
  Fusion protein
MTSSHAMNITPLAQLALLFSTLLLPGTQALLAPTTPDAGSALNLTFDPWTRTLTWACDTAAGNVTVTSCTVTSREAGIHRRVSPFGCRCWFRRMMALHHGVTLDVNGTVGGAAAHWRLSFVNEGAAGSGAENLTCEIRAARFLSCAWREGPAAPADVRYSLRVLNSTGHDVARCMADPGDDVITQCIANDLSLLGSEAYLVVTGRSGAGPVRFLDDVVATKALERLGPPRDVTASCNSSHCTVSWAPPSTWASLTARDFQFEVQWQSAEPGSTPRKVLVVEETRLAFPSPAPHGGHKVKVRAGDTRMKHWGEWSPAHPLEAEDTRVPPSLFALEAVLIPVGTMGLIITLIFVYCWLERMPPIPPIKNLEDLVTEYQGNFSAWSGVSKGLTESLQPDYSERFCHVSEIPPKGGALGEGPGGSPCSLHSPYWPPPCYSLKPEAGSGATNFSLLKQAGDVEENPGPMDQQMALTWGLCYMALVALCWGHGVTEAEETVPLKTLQCYNDYTNHIICSWADTEDAQGLINMTLYHQLEKKQPVSCELSEELMWSECPSSHRCVPRRCVIPYTRFSITNEDYYSFRPDSDLGIQLMVPLAQNVQPPLPKNVSISSSEDRFLLEWSVSLGDAQVSWLSSKDIEFEVAYKRLQDSWEDAYSLHTSKFQVNFEPKLFLPNSIYAARVRTRLSPGSSLSGRPSRWSPEVHWDSQPGDKAQPQNLQCFFDGIQSLHCSWEVWTQTTGSVSFGLFYRPSPVAPEEKCSPVVKEPPGASVYTRYHCSLPVPEPSAHSQYTVSVKHLEQGKFIMSYNHIQMEPPTLNLTKNRDSYSLHWETQKMAYSFIEHTFQVQYKKKSDSWEDSKTENLDRAHSMDLSQLEPDTSYCARVRVKPISNYDGIWSKWSEEYTWKTDWILPMSWLRYLLLVLGCFSGFFSCVYILVKCRYLGPWLKTVLKCHIPDPSEFFSQLSSQHGGDLQKWLSSPVPLSFFSPSGPAPEISPLEVLDGDSKAVQLLLLQKDSAPLPSPSGHSQASCFTNQGYFFFHLPNALEIESCQVYFTYDPCVEEEVEEDGSRLPEGSPHPPLLPLAGEQDDYCAFPPRDDLLLFSPSLSTPNTAYGGSRAPEERSPLSLHEGLPSLASRDLMGLQRPLERMPEGDGEGLSANSSGEQASVPEGNLHGQDQDRGQGPILTLNTDAYLSLQELQAQDSVHLI

SEQ ID NO: 6 - DNA, 1308 bp, Artificial Sequence
  Fusion sequence
atgcttctcctggtgacaagccttctgctctgtgagttaccacacccagcattcctcctgatcccagagaaatcggatctgcgaacagtggcaccagcctctagtctcaatgtgaggtttgactccaggacgatgaatttaagctgggactgccaagaaaacacaaccttcagcaagtgtttcttaactgacaagaagaacagagtcgtggaacccaggctcagtaacaacgaatgttcgtgcacatttcgtgaaatttgtctgcatgaaggagtcacatttgaggttcacgtgaatactagtcaaagaggatttcaacagaaactgctttatccaaattcaggaagggagggtaccgctgctcagaatttctcctgtttcatctacaatgcggatttaatgaactgtacctgggcgaggggtccgacggccccccgtgacgtccagtattttttgtacatacgaaactcaaagagaaggagggagatccggtgtccttattacatacaagactcaggaacccatgtgggatgtcacctggataacctgtcaggattaacgtctcgcaattactttctggttaacggaaccagccgagaaattggcatccaattctttgattcacttttggacacaaagaaaatagaacgattcaaccctcccagcaatgtcaccgtacgttgcaacacgacgcactgcctcgtacggtggaaacagcccaggacctatcagaagctgtcgtacctggactttcagtaccagctggacgtccacagaaagaatacccagcctggcacggaaaacctactgattaatgtttctggtgatttggaaaatagatacaactttccaagctctgagcccagagcaaaacacagtgtgaagatcagagctgcagacgtccgcatcttgaattggagctcctggagtgaagccattgaatttggttctgacgacgggcctttcctgtttgcattggaagccgtggttatctctgttggctccatgggattgattatcagccttctctgtgtgtatttctggctggaacggacgatgccccgaattcccaccctgaagaacctagaggatcttgttactgaataccacgggaacttttcggcctggagtggtgtgtctaagggactggctgagagtctgcagccagactacagtgaacgactctgcctcgtcagtgagattcccccaaaaggaggggcccttggggaggggcctggggcctccccatgcaaccagcatagcccctactgggcccccccatgttacaccctaaagcctgaaacctga

SEQ ID NO: 7 - DNA, 2250 bp, Artificial Sequence
  Fusion sequence
atggtgctggcccaggggctgctctccatggccctgctggccctgtgctgggagcgcagcctggcaggggcagaagaaaccatcccgctgcagaccctgcgctgctacaacgactacaccagccacatcacctgcaggtgggcagacacccaggatgcccagcggctcgtcaacgtgaccctcattcgccgggtgaatgaggacctcctggagccagtgtcctgtgacctcagtgatgacatgccctggtcagcctgcccccatccccgctgcgtgcccaggagatgtgtcattccctgccagagttttgtcgtcactgacgttgactacttctcattccaaccagacaggcctctgggcacccggctcaccgtcactctgacccagcatgtccagcctcctgagcccagggacctgcagatcagcaccgaccaggaccacttcctgctgacctggagtgtggcccttgggagtccccagagccactggttgtccccaggggatctggagtttgaggtggtctacaagcggcttcaggactcttgggaggacgcagccatcctcctctccaacacctcccaggccaccctggggccagagcacctcatgcccagcagcacctacgtggcccgagtacggacccgcctggccccaggttctcggctctcaggacgtcccagcaagtggagcccagaggtttgctgggactcccagccaggggatgaggcccagccccagaacctggagtgcttctttgacggggccgccgtgctcagctgctcctgggaggtgaggaaggaggtggccagctcggtctcctttggcctattctacaagcccagcccagatgcaggggaggaagagtgctccccagtgctgagggaggggctcggcagcctccacaccaggcaccactgccagattcccgtgcccgaccccgcgacccacggccaatacatcgtctctgttcagccaaggagggcagagaaacacataaagagctcagtgaacatccagatggcccctccatccctcaacgtgaccaaggatggagacagctacagcctgcgctgggaaacaatgaaaatgcgatacgaacacatagaccacacatttgagatccagtacaggaaagacacggccacgtggaaggacagcaagaccgagaccctccagaacgcccacagcatggccctgccagccctggagccctccaccaggtactgggccagggtgagggtcaggacctcccgcaccggctacaacgggatctggagcgagtggagtgaggcgcgctcctgggacaccgagtcgattccgtggctcggccacctcctcgtgggcctcagcggggcttttggcttcatcatcttagtgtacttgctgatcaactgcaggaacaccgggccatggctgaagaaggtcctgaagtgtaacaccccagacccctcgaagttcttttcccagctgagctcagagcatggaggagacgtccagaagtggctctcttcgcccttcccctcatcgtccttcagccctggcggcctggcacctgagatctcgccactagaagtgctggagagggacaaggtgacgcagctgctcctgcagcaggacaaggtgcctgagcccgcatccttaagcagcaaccactcgctgaccagctgcttcaccaaccagggttacttcttcttccacctcccggatgccttggagatagaggcctgccaggtgtactttacttacgacccctactcagaggaagaccctgatgagggtgtggccggggcacccacagggtcttccccccaacccctgcagcctctgtcaggggaggacgacgcctactgcaccttcccctccagggatgacctgctgctcttctcccccagtctcctcggtggccccagccccccaagcactgcccctgggggcagtggggccggtgaagagaggatgcccccttctttgcaagaaagagtccccagagactgggacccccagcccctggggcctcccaccccaggagtcccagacctggtggattttcagccaccccctgagctggtgctgcgagaggctggggaggaggtccctgacgctggccccagggagggagtcagtttcccctggtccaggcctcctgggcagggggagttcagggcccttaatgctcgcctgcccctgaacactgatgcctacttgtccctccaagaactccagggtcaggacccaactcacttggtgtag

SEQ ID NO: 8 - DNA, 3637 bp, Artificial Sequence
  Fusion sequence
atgaccagcagccacgccatgaacatcacccccctggctcagctggccctgctgttctctacactgctgctgcctggcacccaggcactgctggctcctacaacacctgatgccggcagcgccctgaacctgaccttcgacccttggaccagaaccctgacctgggcctgtgataccgccgctggcaacgtgaccgtgaccagctgtaccgtgacctccagagaggccggcatccacagaagagtgtccccattcggctgcagatgctggttcagacggatgatggccctgcaccacggcgtgaccctggacgtgaacggaacagtgggcggagccgccgctcattggagactgagctttgtgaacgagggcgcagctggctctggcgccgagaatctgacctgcgagatcagagccgccagattcctgagctgcgcttggagagagggacctgccgctcctgctgacgtgcggtactctctgagagtgctgaacagcaccggccacgatgtggccagatgcatggctgaccctggcgacgacgtgatcacccagtgtatcgccaacgacctgagcctgctgggcagcgaggcttacctggtcgtgacaggcagatctggcgctggcccagtgcggttcctggatgatgtggtggccacaaaggccctggaaagactgggccctcctagggacgtgaccgccagctgtaacagctcccactgcaccgtgtcttgggcccctccatctacatgggccagcctgacagccagagacttccagttcgaagtgcagtggcagagcgccgagcctggcagcacacctagaaaggtgctggtggtggaagagacaagactggccttccccagccctgctcctcacggcggacacaaagtgaaagtgcgggctggcgacaccagaatgaagcactggggagagtggtcccccgctcaccctctggaagccgaggacacaagagtgccccctagcctgttcgccctggaagctgtgctgatccccgtgggcacaatgggcctgatcatcaccctgatcttcgtgtactgttggctggaaagaatgccccccatcccccctatcaagaacctggaagatctcgtgaccgagtaccagggcaacttctccgcttggagcggcgtgtccaagggcctgacagagagcctgcagcccgactacagcgagagattctgccacgtgtccgagatcccccccaagggcggagcactgggagaaggacctggcggcagtccttgtagcctgcacagcccttactggcccccaccctgctacagcctgaagcctgaggctggttccggagccacgaacttctctctgttaaagcaagcaggagacgtggaagaaaaccccggtcccatggatcagcagatggctctgacatggggcctgtgctacatggccctggtggctctgtgttggggccatggcgtgacagaggccgaggaaaccgtgcccctgaaaaccctgcagtgttacaacgactacaccaatcacatcatctgtagctgggccgacaccgaggatgcccagggactgatcaacatgaccctgtaccaccagctggaaaagaaacagcccgtgtcctgcgagctgagcgaggaactgatgtggagcgagtgccctagcagccacagatgtgtgcctagaagatgcgtgatcccctacaccagattcagcatcaccaacgaggactactacagcttcagacccgacagcgacctgggaatccagctgatggtgcccctggcccagaacgtgcagcctcccctgcctaagaacgtgtccatcagcagcagcgaggaccggttcctgctggaatggagtgtgtctctgggcgacgctcaggtgtcctggctgagcagcaaggacatcgagttcgaggtggcctacaagaggctgcaggacagctgggaggacgcctactctctgcacaccagcaagttccaagtgaacttcgagcccaagctgttcctgcccaacagcatctacgccgccagagtgcggaccagactgagccctggatctagcctgagcggcagacctagcagatggtcccctgaggtgcactgggacagccagcctggcgataaggctcagcctcagaacctgcagtgcttcttcgacggcatccagtccctgcactgcagctgggaagtgtggacccagaccacaggcagcgtgtccttcggcctgttctacagaccaagccccgtggcccccgaagagaagtgtagccctgtcgtgaaagagcccccaggcgccagcgtgtacacaagataccactgcagcctgcccgtgcccgagccttctgctcactctcagtacaccgtgtccgtgaagcacctggaacagggcaagttcatcatgagctacaaccacatccagatggaaccccccacactgaatctgacaaagaacagagacagctactccctgcattgggagacacagaagatggcctacagctttatcgagcacacatttcaggtgcagtacaagaagaagtccgactcttgggaggacagcaagaccgaaaacctggacagagcccacagcatggacctgagtcagctggaacccgacaccagctactgtgcccgcgtcagagtgaagcccatcagcaactacgatggcatctggtctaagtggagcgaagagtacacctggaaaaccgactggatcctgcccatgagctggctgagatacctgctgctggtgctgggctgcttcagcggcttcttcagctgcgtgtacatcctcgtgaagtgcagatacctgggcccctggctgaaaaccgtgctgaagtgccacatccccgaccccagcgagttctttagccagctgtctagccagcacggcggcgacctgcagaagtggctgagttctcctgtgcctctgagcttcttctccccctccggacctgcccctgagatcagcccactggaagtgctggacggcgacagcaaggcagtgcagcttctgctgctgcagaaagacagcgcccctctgcctagccctagcggacatagccaggcctcttgctttaccaaccagggctactttttctttcatctgcccaacgctctggaaatcgagagctgtcaggtgtacttcacctacgacccctgcgtggaagaggaagtggaagaggacggcagcagactgcctgagggctctcctcatcctcctctgctgcctctggctggcgagcaggacgactactgcgctttcccaccaagggacgatctgctgctgtttagccccagcctgagcacccccaacaccgcttacggcggaagcagagcccccgaggaaagaagccctctgtctctgcacgagggcctgccttctctggccagcagagatctgatgggcctgcagcggcctctggaacggatgcctgaaggggatggcgagggactgagcgccaactctagcggagagcaggcctctgtgccagagggcaatctgcacggccaggaccaggatagaggccagggcccaatcctgaccctgaacaccgatgcctatctgagtctgcaggaactgcaggcacaggactccgtgcacctgatctgagacccagctttcttgtacaaagtgg

SEQ ID NO: 9 - protein, 320 aa, Homo sapiens
MLLLVTSLLLCELPHPAFLLIPEKSDLRTVAPASSLNVRFDSRTMNLSWDCQENTTFSKCFLTDKKNRVVEPRLSNNECSCTFREICLHEGVTFEVHVNTSQRGFQQKLLYPNSGREGTAAQNFSCFIYNADLMNCTWARGPTAPRDVQYFLYIRNSKRRREIRCPYYIQDSGTHVGCHLDNLSGLTSRNYFLVNGTSREIGIQFFDSLLDTKKIERFNPPSNVTVRCNTTHCLVRWKQPRTYQKLSYLDFQYQLDVHRKNTQPGTENLLINVSGDLENRYNFPSSEPRAKHSVKIRAADVRILNWSSWSEAIEFGSDDG

SEQ ID NO: 10 - protein, 115 aa, Homo sapiens
PFLFALEAVVISVGSMGLIISLLCVYFWLERTMPRIPTLKNLEDLVTEYHGNFSAWSGVSKGLAESLQPDYSERLCLVSEIPPKGGALGEGPGASPCNQHSPYWAPPCYTLKPET

SEQ ID NO: 11 - protein, 438 aa, Homo sapiens
MVLAQGLLSMALLALCWERSLAGAEETIPLQTLRCYNDYTSHITCRWADTQDAQRLVNVTLIRRVNEDLLEPVSCDLSDDMPWSACPHPRCVPRRCVIPCQSFVVTDVDYFSFQPDRPLGTRLTVTLTQHVQPPEPRDLQISTDQDHFLLTWSVALGSPQSHWLSPGDLEFEVVYKRLQDSWEDAAILLSNTSQATLGPEHLMPSSTYVARVRTRLAPGSRLSGRPSKWSPEVCWDSQPGDEAQPQNLECFFDGAAVLSCSWEVRKEVASSVSFGLFYKPSPDAGEEECSPVLREGLGSLHTRHHCQIPVPDPATHGQYIVSVQPRRAEKHIKSSVNIQMAPPSLNVTKDGDSYSLRWETMKMRYEHIDHTFEIQYRKDTATWKDSKTETLQNAHSMALPALEPSTRYWARVRVRTSRTGYNGIWSEWSEARSWDTES

SEQ ID NO: 12 - protein, 311 aa, Homo sapiens
IPWLGHLLVGLSGAFGFIILVYLLINCRNTGPWLKKVLKCNTPDPSKFFSQLSSEHGGDVQKWLSSPFPSSSFSPGGLAPEISPLEVLERDKVTQLLLQQDKVPEPASLSSNHSLTSCFTNQGYFFFHLPDALEIEACQVYFTYDPYSEEDPDEGVAGAPTGSSPQPLQPLSGEDDAYCTFPSRDDLLLFSPSLLGGPSPPSTAPGGSGAGEERMPPSLQERVPRDWDPQPLGPPTPGVPDLVDFQPPPELVLREAGEEVPDAGPREGVSFPWSRPPGQGEFRALNARLPLNTDAYLSLQELQGQDPTHLV

SEQ ID NO: 13 - protein, 22 aa, Artificial Sequence
  Porcine teschovirus-1 2A (P2A) peptide
GSGATNFSLLKQAGDVEENPGP

SEQ ID NO: 14 - protein, 21 aa, Artificial Sequence
  Thoseaasigna virus 2A (T2A) peptide
GSGEGRGSLLTCGDVEENPGP

SEQ ID NO: 15 - protein, 23 aa, Artificial Sequence
  Equine rhinitis A virus (ERAV) 2A (E2A) peptide
GSGQCTNYALLKLAGDVESNPGP

SEQ ID NO: 16 - protein, 25 aa, Artificial Sequence
  Foot-and-Mouth disease virus 2A (F2A) peptide
GSGVKQTLNFDLLKLAGDVESNPGP

SEQ ID NO: 17 - DNA, 66 bp, Artificial Sequence
  Porcine teschovirus-1 2A (P2A) peptide
ggaagcggagctactaacttcagcctgctgaagcaggctggagacgtggaggagaaccctggacct

SEQ ID NO: 18 - DNA, 66 bp, Artificial Sequence
  Porcine teschovirus-1 2A (P2A) peptide - Codon Optimized
ggttccggagccacgaacttctctctgttaaagcaagcaggagacgtggaagaaaaccccggtccc

SEQ ID NO: 19 - DNA, 63 bp, Artificial Sequence
  Thoseaasigna virus 2A (T2A) peptide
ggaagcggagagggcagaggaagtctgctaacatgcggtgacgtcgaggagaatcctggacct

SEQ ID NO: 20 - DNA, 69 bp, Artificial Sequence
  Equine rhinitis A virus (ERAV) 2A (E2A) peptide
ggaagcggacagtgtactaattatgctctcttgaaattggctggagatgttgagagcaaccctggacct

SEQ ID NO: 21 - DNA, 75 bp, Artificial Sequence
  Foot-and-Mouth disease virus 2A (F2A) peptide
ggaagcggagtgaaacagactttgaattttgaccttctcaagttggcgggagacgtggagtccaaccctggacct

SEQ ID NO: 22 - protein, 26 aa, Artificial Sequence
  CSF2RA Transmembrane domain
NLGSVYIYVLLIVGTLVCGIVLGFLF

SEQ ID NO: 23 - protein, 17 aa, Artificial Sequence
  CSF2RB Transmembrane domain
VLALIVIFLTIAVLLAL